European Patent Specification EP 3 197 501 B1, published April 10, 2024. Title: Biological materials and uses thereof. Applicant: Antikor Biopharma Limited. Application PCT/GB2015/052800. The sequence listing filed with the application follows.

SEQUENCE LISTING (8 sequences)

SEQ ID NO: 1 - DNA, 816 bp, Artificial Sequence
  source 1..816: /mol_type="unassigned DNA" /note="DNA sequence of cleaved TCT" /organism="Artificial Sequence"
agcggtagcggaggtagcggacaggtgcagctggtgcagtctggggcagaggtgaaaaagcccggggagtctctgaagatctcctgtaagggttctggatacagctttaccagctactggatcgcctgggtgcgccagatgcccgggaaaggcctggagtacatggggctcatctatcctggtgactctgacaccaaatacagcccgtccttccaaggccaggtcaccatctcagtcgacaagtccgtcagcactgcctacttgcaatggagcagtctgaagccctcggacagcgccgtgtatttttgtgcgagacatgacgtgggatattgcagtagttccaactgcgcagcgtggcctgaatacttccagcattggggccagggcaccctggtcaccgtctcctcaggtggaggcggttcaggcggaggtggctctggcggtggcggatcgcagtctgtgttgacgcagccgccctcagtgtctgcggccccaggacagaaggtcaccatctcctgctctggaagcagctccaacattgggaataattatgtatcctggtaccagcagctcccaggaacagcccccaaactcctcatctatggtcacaccaatcggcccgcaggggtccctgaccgattctctggctccaagtctggcacctcagcctccctggccatcagtgggttccggtccgaggatgaggctgattattactgtgcagcatgggatgacagcctgagtggttgggtgttcggcggagggaccaagctgaccgtcctaatggctagcatgactggtggacagcaaatgggt

SEQ ID NO: 2 - protein, 272 aa, Artificial Sequence
  Amino Acid sequence of cleaved TCT
SGSGGSGQVQLVQSGAEVKKPGESLKISCKGSGYSFTSYWIAWVRQMPGKGLEYMGLIYPGDSDTKYSPSFQGQVTISVDKSVSTAYLQWSSLKPSDSAVYFCARHDVGYCSSSNCAAWPEYFQHWGQGTLVTVSSGGGGSGGGGSGGGGSQSVLTQPPSVSAAPGQKVTISCSGSSSNIGNNYVSWYQQLPGTAPKLLIYGHTNRPAGVPDRFSGSKSGTSASLAISGFRSEDEADYYCAAWDDSLSGWVFGGGTKLTVLMASMTGGQQMG

SEQ ID NO: 3 - DNA, 838 bp, Artificial Sequence
  source 1..838: /mol_type="unassigned DNA" /note="DNA sequence of cleaved TCT1067 " /organism="Artificial Sequence"
gcggtagcggaggtagcggacaggtgcagctggtgcagtctggggcagaggtgaaaaagcccggggagtctctgaagatctcctgtaagggttctggatacagctttaccagctactggatcgcctgggtgcgccagatgcccgggaaaggcctggagtacatggggctcatctatcctggtgactctgacaccaaatacagcccgtccttccaaggccaggtcaccatctcagtcgacaagtccgtcagcactgcctacttgcaatggagcagtctgaagccctcggacagcgccgtgtatttttgtgcgagacatgacgtgggatattgcaccgatcgtacctgcgcagcgtggcctgaatggctgggcgtgtggggccagggcaccctggtcaccgtctcctcaggtggaggcggttcaggcggaggtggctctggcggtggcggatcgcagtctgtgttgacgcagccgccctcagtgtctgcggccccaggacagaaggtcaccatctcctgctctggaagcagctccaacattgggaataattatgtatcctggtaccagcagctcccaggaacagcccccaaactcctcatctatggtcacaccaatcggcccgcaggggtccctgaccgattctctggctccaagtctggcacctcagcctccctggccatcagtgggttccggtccgaggatgaggctgattattactgtgcaagctgggattataccctgagtggttgggtgttcggcggagggaccaagctgaccgtcctaatggctagcatgactggtggacagcaaatgggttgatgaggctctaactctcctct

SEQ ID NO: 4 - protein, 272 aa, Artificial Sequence
  Amino Acid sequence of cleaved scFv (TCT1067)
SGSGGSGQVQLVQSGAEVKKPGESLKISCKGSGYSFTSYWIAWVRQMPGKGLEYMGLIYPGDSDTKYSPSFQGQVTISVDKSVSTAYLQWSSLKPSDSAVYFCARHDVGYCTDRTCAAWPEWLGVWGQGTLVTVSSGGGGSGGGGSGGGGSQSVLTQPPSVSAAPGQKVTISCSGSSSNIGNNYVSWYQQLPGTAPKLLIYGHTNRPAGVPDRFSGSKSGTSASLAISGFRSEDEADYYCASWDYTLSGWVFGGGTKLTVLMASMTGGQQMG

SEQ ID NO: 5 - protein, 257 aa, Artificial Sequence
  Amino acid sequence of panitumumab single chain Fv
QVQLQESGPGLVKPSETLSLTCTVSGGSVSSGDYYWTWIRQSPGKGLEWIGHIYYSGNTNYNPSLKSRLTISIDTSKTQFSLKLSSVTAADTAIYYCVRDRVTGAFDIWGQGTMVTVSSGGGGSGGGGSGGGGSDIQMTQSPSSLSASVGDRTVITCQASQDISNYLNWYQQKPGKAPKLLIYDASNLETGVPSRFSGSGSGTDFTFTISSLQPEDIATYFCQHFDHLPLAFGGGTKVEIQNGSEQKLISEEDLAAA

SEQ ID NO: 6 - protein, 254 aa, Artificial Sequence
  Amino acid sequence of scFv (TCT1067)
QVQLVQSGAEVKKPGESLKISCKGSGYSFTSYWIAWVRQMPGKGLEYMGLIYPGDSDTKYSPSFQGQVTISVDKSVSTAYLQWSSLKPSDSAVYFCARHDVGYCTDRTCAAWPEWLGVWGQGTLVTVSSGGGGSGGGGSGGGGSQSVLTQPPSVSAAPGQKVTISCSGSSSNIGNNYVSWYQQLPGTAPKLLIYGHTNRPAGVPDRFSGSKSGTSASLAISGFRSEDEADYYCASWDYTLSGWVFGGGTKLTVL

SEQ ID NO: 7 - protein, 241 aa, Artificial Sequence
  Amino acid sequence of scFv (panitumumab)
QVQLQESGPGLVKPSETLSLTCTVSGGSVSSGDYYWTWIRQSPGKGLEWIGHIYYSGNTNYNPSLKSRLTISIDTSKTQFSLKLSSVTAADTAIYYCVRDRVTGAFDIWGQGTMVTVSSGGGGSGGGGSGGGGSDIQMTQSPSSLSASVGDRTVITCQASQDISNYLNWYQQKPGKAPKLLIYDASNLETGVPSRFSGSGSGTDFTFTISSLQPEDIATYFCQHFDHLPLAFGGGTKVEIQ

SEQ ID NO: 8 - protein, 6 aa, Artificial Sequence
  Linker region
GSGGSG